European Patent Application EP 4 397 684 A1, published July 10, 2024. Title: ANTI-HUMAN TSLP MONOCLONAL ANTIBODY AND USE THEREOF. Applicant: Qyuns Therapeutics Co., Ltd. The sequence listing filed with the application follows.

SEQUENCE LISTING (11 sequences)

SEQ ID NO: 1 - protein, 5 aa, Artificial sequence
  Description of Artificial Sequence: artificially synthesized sequence
SYYMS

SEQ ID NO: 2 - protein, 16 aa, Artificial sequence
  Description of Artificial Sequence: artificially synthesized sequence
FISYGGSAYHATWAQG

SEQ ID NO: 3 - protein, 13 aa, Artificial sequence
  Description of Artificial Sequence: artificially synthesized sequence
EFRSMTYGAEWGI

SEQ ID NO: 4 - protein, 11 aa, Artificial sequence
  Description of Artificial Sequence: artificially synthesized sequence
QASESIYDTLA

SEQ ID NO: 5 - protein, 7 aa, Artificial sequence
  Description of Artificial Sequence: artificially synthesized sequence
SASSLAS

SEQ ID NO: 6 - protein, 13 aa, Artificial sequence
  Description of Artificial Sequence: artificially synthesized sequence
QQGYTMPDVDKNP

SEQ ID NO: 7 - protein, 121 aa, Artificial sequence
  Description of Artificial Sequence: artificially synthesized sequence
EVQLVESGGGLVQPGGSLRLSCAASGFSLSSYYMSWVRQAPGKGLEWVGFISYGGSAYHATWAQGRFTISKDNSKNTLYLQMNSLRAEDTAVYYCAREFRSMTYGAEWGIWGQGTLVTVSS

SEQ ID NO: 8 - protein, 111 aa, Artificial sequence
  Description of Artificial Sequence: artificially synthesized sequence
AYQMTQSPSSVSASVGDRVTITCQASESIYDTLAWYQQKPGKAPKLLIYSASSLASGVPSRFSGSGSGTDFTLTISSLQPEDFATYYCQQGYTMPDVDKNPFGGGTKVEIK

SEQ ID NO: 9 - protein, 159 aa, Artificial sequence
  Description of Artificial Sequence: artificially synthesized sequence
MFPFALLYVLSVSFRKIFILQLVGLVLTYDFTNCDFEKIKAAYLSTISKDLITYMSGTKSTEFNNTVSCSNRPHCLTEIQSLTFNPTAGCASLAKEMFAMKTKAALAIWCPGYSETQINATQAMKKRRKRKVTTNKCLEQVSQLQGLWRRFNRPLLKQQ

SEQ ID NO: 10 - protein, 451 aa, Artificial sequence
  Description of Artificial Sequence: artificially synthesized sequence
EVQLVESGGGLVQPGGSLRLSCAASGFSLSSYYMSWVRQAPGKGLEWVGFISYGGSAYHATWAQGRFTISKDNSKNTLYLQMNSLRAEDTAVYYCAREFRSMTYGAEWGIWGQGTLVTVSSASTKGPSVFPLAPSSKSTSGGTAALGCLVKDYFPEPVTVSWNSGALTSGVHTFPAVLQSSGLYSLSSVVTVPSSSLGTQTYICNVNHKPSNTKVDKKVEPKSCDKTHTCPPCPAPELLGGPSVFLFPPKPKDTLMISRTPEVTCVVVDVSHEDPEVKFNWYVDGVEVHNAKTKPREEQYNSTYRVVSVLTVLHQDWLNGKEYKCKVSNKALPAPIEKTISKAKGQPREPQVYTLPPSRDELTKNQVSLTCLVKGFYPSDIAVEWESNGQPENNYKTTPPVLDSDGSFFLYSKLTVDKSRWQQGNVFSCSVMHEALHNHYTQKSLSLSPGK

SEQ ID NO: 11 - protein, 218 aa, Artificial sequence
  Description of Artificial Sequence: artificially synthesized sequence
AYQMTQSPSSVSASVGDRVTITCQASESIYDTLAWYQQKPGKAPKLLIYSASSLASGVPSRFSGSGSGTDFTLTISSLQPEDFATYYCQQGYTMPDVDKNPFGGGTKVEIKRTVAAPSVFIFPPSDEQLKSGTASVVCLLNNFYPREAKVQWKVDNALQSGNSQESVTEQDSKDSTYSLSSTLTLSKADYEKHKVYACEVTHQGLSSPVTKSFNRGEC